European Patent Application EP 4 624 581 A1, published October 1, 2025. Title: MICROORGANISMS FOR PRODUCING PURINE NUCLEOTIDES AND PROCESS FOR PRODUCING PURINE NUCLEOTIDES USING THE SAME. Applicant: CJ CheilJedang Corporation. The sequence listing filed with the application follows.

SEQUENCE LISTING (83 sequences)

SEQ ID NO: 1 - DNA, 35 bp, synthetic construct
  source 1..35: mol_type = other DNA
acccggggatcctctagagtgccgttacctcccgc

SEQ ID NO: 2 - DNA, 36 bp, synthetic construct
  source 1..36: mol_type = other DNA
tggagtgcgtagcgtgcgaaatgactcctttctaaa

SEQ ID NO: 3 - DNA, 36 bp, synthetic construct
  source 1..36: mol_type = other DNA
tttagaaaggagtcatttcgcacgctacgcactcca

SEQ ID NO: 4 - DNA, 36 bp, synthetic construct
  source 1..36: mol_type = other DNA
aagcttgcatgcctgcagcgtcaccgcgcggagata

SEQ ID NO: 5 - DNA, 25 bp, synthetic construct
  source 1..25: mol_type = other DNA
gaaatgactcctttctaaaaagggg

SEQ ID NO: 6 - DNA, 39 bp, synthetic construct
  source 1..39: mol_type = other DNA
ttagaaaggagtcatttcgaacttgcagcaaacgtgctg

SEQ ID NO: 7 - DNA, 20 bp, synthetic construct
  source 1..20: mol_type = other DNA
ccttggtgaggcactttgtg

SEQ ID NO: 8 - DNA, 39 bp, synthetic construct
  source 1..39: mol_type = other DNA
caaagtgcctcaccaagggcacgctacgcactccatata

SEQ ID NO: 9 - DNA, 20 bp, synthetic construct
  source 1..20: mol_type = other DNA
gtcaacgcgcacttggatct

SEQ ID NO: 10 - DNA, 38 bp, synthetic construct
  source 1..38: mol_type = other DNA
aattcgagctcggtacccaggcacagccgacattacgg

SEQ ID NO: 11 - DNA, 35 bp, synthetic construct
  source 1..35: mol_type = other DNA
gtagcacatctgacgaatgtccaagtctaaggaaa

SEQ ID NO: 12 - DNA, 35 bp, synthetic construct
  source 1..35: mol_type = other DNA
ttagacttggacattcgtcagatgtgctacttgcc

SEQ ID NO: 13 - DNA, 35 bp, synthetic construct
  source 1..35: mol_type = other DNA
tgcgccattagcgtgttacttctcgcggctataga

SEQ ID NO: 14 - DNA, 35 bp, synthetic construct
  source 1..35: mol_type = other DNA
agccgcgagaagtaacacgctaatggcgcattgaa

SEQ ID NO: 15 - DNA, 35 bp, synthetic construct
  source 1..35: mol_type = other DNA
tgaattatccgcgtcttagatgccgttttctgccg

SEQ ID NO: 16 - DNA, 35 bp, synthetic construct
  source 1..35: mol_type = other DNA
gaaaacggcatctaagacgcggataattcagctgt

SEQ ID NO: 17 - DNA, 38 bp, synthetic construct
  source 1..38: mol_type = other DNA
cgactctagaggatccccgatgaagcgaacacttaaat

SEQ ID NO: 18 - DNA, 20 bp, synthetic construct
  source 1..20: mol_type = other DNA
ccagtacattgtcatgggat

SEQ ID NO: 19 - DNA, 20 bp, synthetic construct
  source 1..20: mol_type = other DNA
gattggcatatcgcaccgag

SEQ ID NO: 20 - DNA, 38 bp, synthetic construct
  source 1..38: mol_type = other DNA
tcgagctcggtacccgttgccgtatcagacatgctcag

SEQ ID NO: 21 - DNA, 38 bp, synthetic construct
  source 1..38: mol_type = other DNA
gattagcctgaaggaattgatttatctcgaccaaacag

SEQ ID NO: 22 - DNA, 38 bp, synthetic construct
  source 1..38: mol_type = other DNA
ggtcgagataaatcaattccttcaggctaatcttttcc

SEQ ID NO: 23 - DNA, 38 bp, synthetic construct
  source 1..38: mol_type = other DNA
cgatataagactccatcatatgtgtttcctttcgttgg

SEQ ID NO: 24 - DNA, 38 bp, synthetic construct
  source 1..38: mol_type = other DNA
aaaggaaacacatatgatggagtcttatatcggtagcc

SEQ ID NO: 25 - DNA, 38 bp, synthetic construct
  source 1..38: mol_type = other DNA
ctcataggtgccgaacttactcggagatttcgacctca

SEQ ID NO: 26 - DNA, 38 bp, synthetic construct
  source 1..38: mol_type = other DNA
cgaaatctccgagtaagttcggcacctatgagaatatg

SEQ ID NO: 27 - DNA, 39 bp, synthetic construct
  source 1..39: mol_type = other DNA
ctctagaggatccccggcaagtgtttcttggcgccattc

SEQ ID NO: 28 - DNA, 20 bp, synthetic construct
  source 1..20: mol_type = other DNA
taatcccccagctcaccggc

SEQ ID NO: 29 - DNA, 20 bp, synthetic construct
  source 1..20: mol_type = other DNA
tttggatgccgaggtcgtag

SEQ ID NO: 30 - DNA, 38 bp, synthetic construct
  source 1..38: mol_type = other DNA
aattcgagctcggtaccccatttcgtgaccattagcgt

SEQ ID NO: 31 - DNA, 35 bp, synthetic construct
  source 1..35: mol_type = other DNA
ctttgtacttggtgagatcatgccaatagcgccag

SEQ ID NO: 32 - DNA, 35 bp, synthetic construct
  source 1..35: mol_type = other DNA
gctattggcatgatctcaccaagtacaaagagact

SEQ ID NO: 33 - DNA, 38 bp, synthetic construct
  source 1..38: mol_type = other DNA
cgactctagaggatccccggttaccgcgcattaggact

SEQ ID NO: 34 - DNA, 20 bp, synthetic construct
  source 1..20: mol_type = other DNA
taatcccccagctcaccggc

SEQ ID NO: 35 - DNA, 20 bp, synthetic construct
  source 1..20: mol_type = other DNA
tttggatgccgaggtcgtag

SEQ ID NO: 36 - DNA, 38 bp, synthetic construct; identical to SEQ ID NO: 30
  source 1..38: mol_type = other DNA

SEQ ID NO: 37 - DNA, 35 bp, synthetic construct
  source 1..35: mol_type = other DNA
attagcctgaaggaagatcatgccaatagcgccag

SEQ ID NO: 38 - DNA, 35 bp, synthetic construct
  source 1..35: mol_type = other DNA
gctattggcatgatcttccttcaggctaatctttt

SEQ ID NO: 39 - DNA, 35 bp, synthetic construct
  source 1..35: mol_type = other DNA
attctgggtagtcatcatatgtgtttcctttcgtt

SEQ ID NO: 40 - DNA, 35 bp, synthetic construct
  source 1..35: mol_type = other DNA
aaggaaacacatatgatgactacccagaattcttc

SEQ ID NO: 41 - DNA, 35 bp, synthetic construct
  source 1..35: mol_type = other DNA
ctttgtacttggtgaccaagagtcaggatgccgaa

SEQ ID NO: 42 - DNA, 35 bp, synthetic construct
  source 1..35: mol_type = other DNA
catcctgactcttggtcaccaagtacaaagagact

SEQ ID NO: 43 - DNA, 38 bp, synthetic construct; identical to SEQ ID NO: 33
  source 1..38: mol_type = other DNA

SEQ ID NO: 44 - DNA, 20 bp, synthetic construct
  source 1..20: mol_type = other DNA
taatcccccagctcaccggc

SEQ ID NO: 45 - DNA, 20 bp, synthetic construct
  source 1..20: mol_type = other DNA
tttggatgccgaggtcgtag

SEQ ID NO: 46 - DNA, 38 bp, synthetic construct; identical to SEQ ID NO: 10
  source 1..38: mol_type = other DNA

SEQ ID NO: 47 - DNA, 35 bp, synthetic construct; identical to SEQ ID NO: 11
  source 1..35: mol_type = other DNA

SEQ ID NO: 48 - DNA, 35 bp, synthetic construct; identical to SEQ ID NO: 12
  source 1..35: mol_type = other DNA

SEQ ID NO: 49 - DNA, 35 bp, synthetic construct; identical to SEQ ID NO: 13
  source 1..35: mol_type = other DNA

SEQ ID NO: 50 - DNA, 35 bp, synthetic construct; identical to SEQ ID NO: 14
  source 1..35: mol_type = other DNA

SEQ ID NO: 51 - DNA, 35 bp, synthetic construct; identical to SEQ ID NO: 15
  source 1..35: mol_type = other DNA

SEQ ID NO: 52 - DNA, 35 bp, synthetic construct; identical to SEQ ID NO: 16
  source 1..35: mol_type = other DNA

SEQ ID NO: 53 - DNA, 38 bp, synthetic construct; identical to SEQ ID NO: 17
  source 1..38: mol_type = other DNA

SEQ ID NO: 54 - DNA, 20 bp, synthetic construct
  source 1..20: mol_type = other DNA
ccagtacattgtcatgggat

SEQ ID NO: 55 - DNA, 20 bp, synthetic construct
  source 1..20: mol_type = other DNA
gattggcatatcgcaccgag

SEQ ID NO: 56 - DNA, 38 bp, synthetic construct; identical to SEQ ID NO: 20
  source 1..38: mol_type = other DNA

SEQ ID NO: 57 - DNA, 38 bp, synthetic construct; identical to SEQ ID NO: 21
  source 1..38: mol_type = other DNA

SEQ ID NO: 58 - DNA, 38 bp, synthetic construct; identical to SEQ ID NO: 22
  source 1..38: mol_type = other DNA

SEQ ID NO: 59 - DNA, 38 bp, synthetic construct; identical to SEQ ID NO: 23
  source 1..38: mol_type = other DNA

SEQ ID NO: 60 - DNA, 38 bp, synthetic construct; identical to SEQ ID NO: 24
  source 1..38: mol_type = other DNA

SEQ ID NO: 61 - DNA, 38 bp, synthetic construct; identical to SEQ ID NO: 25
  source 1..38: mol_type = other DNA

SEQ ID NO: 62 - DNA, 38 bp, synthetic construct; identical to SEQ ID NO: 26
  source 1..38: mol_type = other DNA

SEQ ID NO: 63 - DNA, 39 bp, synthetic construct; identical to SEQ ID NO: 27
  source 1..39: mol_type = other DNA

SEQ ID NO: 64 - DNA, 19 bp, synthetic construct
  source 1..19: mol_type = other DNA
gcgagggggaagaaaagta

SEQ ID NO: 65 - DNA, 18 bp, synthetic construct
  source 1..18: mol_type = other DNA
cgttgccctttttcttct

SEQ ID NO: 66 - protein, 470 aa, Corynebacterium stationis
VTISVIDIFSVGVGPSSSHTVGPMRAAKTFMESLPHAPAKVHTELRGSLSATGKGHATDRAVILGLAGWAPLTVPIDAKPLAGSFIPSEGTVEGPAGSVQYSIAFNNKPVPEHPNCLIFSAWDENGEEIATNMEYFSVGGGFVLSRAELDAQLQATHEVPAGMAAAQNNDNAIPYDFSTGDQLLELCDEHDMTIWEIVAANEAVIHREDGGLAKVNAHLDLVWDVMRECVTDGIATKGILPGGLQVNRRAPQLYSQLLEHQDDTASGFSAMEWVNLYALAVNEQNAAGGRVVTAPTNGACGIIPAVLHYARDFLPDFTRETARRFLLTAGAIGMIIKQNASISGAEVGCQGEVGSASSMAAAGLAEILGSSPAQIENAAEIALEHNLGLTCDPVGGLVQIPCIERNAIGAVKSINSARLARMGEGTHYVTLDNAVQTMAETGRDMLTKYKETSIGGLAKTLGLSVSQVEC

SEQ ID NO: 67 - DNA, 1413 bp, Corynebacterium stationis
  source 1..1413: mol_type = genomic DNA
gtgaccattagcgtcattgacatcttttcagtaggcgtggggccttcgtcctcccacaccgttggccccatgcgtgcagcgaaaacctttatggaatctttgccgcatgctcctgccaaagtacatactgagctgcgtggttcactctcagccacgggtaaaggccacgccaccgaccgcgccgtcattttaggccttgccggatgggcgccacttaccgtacctattgacgctaagccgcttgccggcagttttatcccttctgaaggcacagtcgaaggccccgccggcagcgtgcagtattccattgcgttcaacaacaagccggtgcctgagcacccgaactgtttgatatttagcgcctgggatgaaaatggtgaagaaatcgctaccaatatggagtacttctccgtgggcggcggctttgttctctcacgtgcagagctcgatgcgcagctgcaagccacccacgaagttccggcgggtatggcggctgcgcaaaataatgacaacgcaatcccctatgacttcagcaccggtgatcagctcctagagttgtgcgatgagcacgacatgacaatctgggaaatcgtcgctgccaatgaagcagttattcaccgtgaagatggtgggctggccaaggtcaacgcgcacttggatctggtgtgggatgtcatgcgtgagtgtgttactgatggcattgctaccaaggggattttgcccggtggtctgcaggttaatcgtcgtgctccgcaactttatagtcaattgcttgaacaccaagatgatactgcgtcaggcttttctgccatggagtgggtcaacctctatgcactagccgtcaacgagcaaaatgctgccggtggccgcgtggtcactgctccaactaacggtgcctgcggaatcattcccgcggtcttgcactatgcacgagacttcctccccgatttcactcgtgagacagcccggcgttttctgctcaccgctggcgctattggcatgatcatcaagcagaatgcttctatctctggcgctgaggttggctgccaaggagaagtcggctcggcatcgtcaatggctgctgccgggttggctgagattttaggctcgagtccagcacagatcgaaaatgcggcagaaatagcactcgagcacaatctcggtctaacctgcgatccggtcggcggcttggtgcagattccgtgcatcgagcgcaatgcgattggcgcagtaaagtctattaactccgcacgccttgcccgcatgggtgaaggcacgcattacgtcaccctcgataatgctgtgcagacaatggccgagaccggccgagacatgctcaccaagtacaaagagacttcgatcggtggcttggctaagaccctgggactatctgtctcccaggtggagtgctaa

SEQ ID NO: 68 - protein, 361 aa, Corynebacterium stationis
MTATTNHLTENSHAHGYDHYQRMAFFTDTSVCIGCKACEVACKEWNRNPVEGYNLTGNSYDNTGALGANTWRHVAFIEQDNERITKAREEGAKLVSLGMPTIGTSPVDAAPNPASADTTPPDTDTFRWLMSSDVCKHCTNAGCLDVCPTGALFRTEFGTVVVQDDVCNGCGTCVAGCPFGVIERREDGGVSLKANHVEAQEVPEHAGINVFKKLKQLRPQGPDHVPGETMPIKNIGVAQKCTMCYDRLKVGEQPACSKTCPTESIQFGTYENMLAAAQARVAELHRQGQTEARLYGANNEDGVGGTGSIFLLLDSPEVYGLPPDPRVPTADLPAMAKTFAKAVGAMGVAVAASFLVDRGGT

SEQ ID NO: 69 - DNA, 1086 bp, Corynebacterium stationis
  source 1..1086: mol_type = genomic DNA
atgacggctacgaccaatcacctaacagaaaattcgcacgcgcacggctacgaccattaccagcgcatggcctttttcaccgatacttcggtgtgcattggctgtaaggcttgcgaggtggcctgtaaggagtggaaccgcaacccggttgagggctataacctgacgggtaattcctacgacaacaccggcgcgctgggcgcgaatacctggcgacacgtagcatttattgagcaagacaacgagcgcatcaccaaagcgcgtgaagaaggtgccaagctggtctcgctgggcatgccgacgattggcacttcgcctgtcgatgcagccccgaatcctgcctccgccgataccacgccgccggatactgatactttccgttggctgatgtcttctgatgtctgcaagcactgcaccaacgctggctgcctggatgtgtgcccaaccggtgctttatttcgcaccgaatttggcaccgtcgtggtccaagatgatgtctgcaatggctgcggcacctgcgttgccgggtgcccgttcggtgttattgagcgccgtgaagacggcggtgtttcgctaaaagccaaccacgtcgaagcccaagaagtccctgaacacgcgggcattaacgtgtttaagaagctcaaacagctgcgcccgcaaggaccggatcacgtcccgggtgagaccatgccgattaaaaatattggcgtggctcaaaagtgcaccatgtgctacgaccgcctgaaagtcggcgagcagccagcgtgttccaagacatgcccgacggagtccatccagttcggcacctatgagaatatgctggccgctgcgcaagcgcgcgtggctgagctacaccgtcaaggccagactgaggcacgactgtacggcgcaaataacgaagacggcgtcggcggaacgggctccatcttcttgctgctggattccccggaagtctacggtcttccaccagatccgcgtgtgccgactgcagatttgcccgcaatggcgaagactttcgccaaggccgttggcgccatgggcgttgccgtggcagcgtcctttttagttgatagaggagggacctag

SEQ ID NO: 70 - protein, 923 aa, Corynebacterium stationis
LGTSFGRGGATQPLQDMANADCILIQGSNMAECHPVGFQWVVEAKKRGARVIHVDPRYTRTSAFANRHVAIRGGTDVVLLGALIKYMIDNDLYFHDYVVNYTNASSIISPDFRDTEDLDGLFSGYNPETGKYITDSWQYVQKPEGAWWNIERDETLQDPNTVFQILKRHYSRYTPEIVEETCGISQEDFHYLAESIAQNSNPERTTVFAYALGFTQQTLGVQFIRAAAILQLLMGNVGRPGSGIMALRGHASIQGSTDIPTLFNNLPGYLPMPHADHGDWKGFLDAIAKEDQKGFWGLRENYAVSLMKSYWGENATKDNDWGWNYMPRINGAHSTYETLMGMLDGIVEGYIVFGQNPAVAQSNGGMQRRGLASLKWLVVRDFQEIETASFWYDSPEIKTGELKTEDIGTEVFLLPAATHVEKAGTFTQTQRMLQWRFQATNPPGDAKSDLWFFYQMGKRIREKLAGSTDPMDAPLLAIDWNYEETEHGEPDPEDVLREINGYYLDGPKKGQLLPGFTEMKPDGTTSGGCWIYSGVFKDNINQSARKVSGASQNEVALEWGWVWPSNRRMLYNRASAAPDGTPWSERKKYIWWDAEAGRWTGDDVPDFPVNLDPSYRAPVDATGPAALDGTDAFIMQADGRGWLFVPKGLSDGPLPTHYEPHESPARNILYSQQQSPTRLTIKRPDNLSKPMAGEPGSEVYPVVFSTYRLTEMYTSGAMSRRLPYLAELQPDLFVEVDPVLAQKRGLENGGWATIISPRGVIEARVLVTERMESMTINGKDFHQIGLPFHYGQSSSSPVTGDGANDLLGLTLEPNVFIQNSKVGACEIKAGRRPRGKARLEMLKEYQRRAGLTLDTGNELIDPDAQQLEATSTIDLFIPNGVDKETVETSTSEPGAADGSAHHGSAMGEVPNSEPKDTEGGEKQ

SEQ ID NO: 71 - DNA, 2772 bp, Corynebacterium stationis
  source 1..2772: mol_type = genomic DNA
ttgggaacctcgtttggccgcggtggcgcaactcagccactgcaggatatggcaaatgccgactgcatcctgattcagggctcgaatatggccgagtgccatcctgtgggtttccagtgggtagtcgaagctaaaaagcgcggggcgcgcgtaattcacgtggatcctcgctatacccgtacctcggcgtttgcgaaccggcacgtagcgatccgtggcggcaccgatgtggtgcttcttggcgcacttatcaagtacatgatcgacaatgatctgtattttcacgactatgtggtcaattacacgaacgcgtcgtcgatcatttctcccgacttccgggacacggaagacctagacggcctcttttctggctacaacccagaaaccggtaagtacatcacggactcgtggcagtacgtgcaaaagcccgaaggtgcgtggtggaatatcgagcgtgatgagactttgcaggacccgaatacggtcttccagattctcaagcgccactattcccgctataccccggaaatcgtggaagagacctgcggtatctcccaggaggacttccattatctagcggagtcgattgcacagaactccaatccagagcgcactacagtctttgcctatgctttgggctttacgcagcaaaccttaggcgtgcagttcattcgtgccgcggccatcttgcaactgctgatgggcaacgtgggccgcccgggctcaggcatcatggcgctgcgtggacacgcttccattcagggctcgacagatatcccgacgctgtttaataacttgccgggttacttgccgatgcctcatgccgaccatggcgactggaaaggattcttggacgcgattgccaaggaagaccagaagggtttctggggtctgcgtgaaaactatgccgtgagcttgatgaagtcctattggggcgagaatgccaccaaggacaatgactggggctggaactacatgccgcgcatcaacggtgcgcactccacctatgaaaccttgatgggcatgctcgacggcatcgtcgaaggctatatcgtcttcggacaaaacccagcggtcgctcaatccaacggcggcatgcaacgccgcggattggcgtctttgaagtggttggttgttcgtgacttccaggaaattgagacagcgtcattctggtacgactcaccagagatcaagactggtgaactcaagaccgaagatattggcaccgaggtcttccttcttcctgcagcaacgcacgtagaaaaggccggtacctttacccaaacccagcgcatgctgcagtggcgtttccaggccacaaatccaccaggcgatgccaagagcgatctgtggttcttctaccagatgggcaagcgcattcgcgaaaagcttgctggttctactgatccgatggacgcgccattgttggccatcgactggaactacgaggaaaccgaacacggcgagccagatcccgaagacgtgctgcgcgaaatcaacggctactatctggatggcccgaagaaggggcagctgctgcctggctttacagagatgaagcctgatggcacgacgtctggtggctgctggatctactccggcgtgttcaaggacaacatcaaccagtccgcgcgcaaagtttcaggcgcttcgcaaaatgaggttgcgctggaatggggctgggtatggccatcgaatcgccgcatgctgtacaaccgtgcgtcagctgcgccagacggcacgccatggtcggagcgcaagaagtacatttggtgggacgctgaggccggccgctggacgggcgacgacgtaccggacttcccagtcaacttggatccgtcataccgcgcgcctgtcgatgccacaggtcctgcagcccttgacggcaccgatgcgtttatcatgcaggcagatggtcgtggttggttgttcgtacccaaaggactttccgatggacccctgccaacccactatgaaccgcacgagtcgccggcacgcaatattttgtacagccagcagcagtcgccgacacgcttgaccatcaagcgtccggataacttgtcgaagcccatggctggtgagcccggctcagaggtctaccccgtggttttctccacgtaccgtttgacggagatgtacacctcgggtgcgatgagccgccgactgccttatttggcagagttgcagccagatttgttcgttgaggtcgatccggttctagcacaaaagcgcggcttggaaaacggtggctgggcaaccatcatttcgccgcgtggcgtgattgaggctcgcgtgctggtgaccgaacgcatggaatctatgaccatcaatggcaaggacttccaccagattggtctgcctttccactacggtcagtccagctcctcgccagttactggtgacggtgccaatgaccttctgggtctaactttggagccgaatgtgttcattcaaaactccaaggttggtgcatgtgaaattaaggccggccgacgcccacgcggcaaggcgcggttagagatgctcaaggaataccagcgccgtgccggattgacgttggacaccggtaacgagctcatcgatcccgatgcacagcagctcgaagctacctccacgatcgacttatttattccgaatggcgtagacaaagagacggtggagacatcgacaagcgagcctggcgccgcagatggttctgcgcatcatggctcagcgatgggggaagtcccaaattctgaaccaaaagatacggagggaggcgaaaagcaatga

SEQ ID NO: 72 - protein, 188 aa, Corynebacterium stationis
MSKLSPLNWPVVRQVKRGDLFGRDKSTQSAKSENLHGRTVEADKVVQSVCPYCAVGCSQRVYVKDDRVVHIEGDSDSPISRGRLCPKGAASEQLVNSATRLTKIKYRAPHATEWQDLDLETAMDMIADRFIASRRNQWQDFDEKGRVLNRTMGVAGLGGATLDNEENYIIKKLFTAAGAVQVENQARI

SEQ ID NO: 73 - DNA, 567 bp, Corynebacterium stationis
  source 1..567: mol_type = genomic DNA
atgtcgaagttaagtccgctgaattggccggttgtgcgccaggtgaagcgcggcgatctgtttggtcgagataaatcaacccagtctgccaaatcggagaacctgcacgggcgcactgtagaggccgacaaagtagttcaatcggtctgcccttactgcgctgtgggctgctcgcagcgggtatatgtcaaagatgaccgcgtcgttcatattgaaggtgactcggactcgcctatttcgcgcggacgtttgtgcccgaaaggcgctgcctctgagcagctggtgaactctgcgacgcgtttgaccaagattaaataccgcgcgcctcatgcaaccgagtggcaagacctagatctcgaaaccgcaatggatatgattgcggaccgttttattgcctcccgccgcaatcagtggcaggactttgatgaaaaaggccgtgttttaaaccgcaccatgggtgtggcaggacttggtggcgccaccttggataatgaggaaaactacattatcaagaagctgtttactgcagctggtgccgtacaagtcgaaaaccaagcacgcatatga

SEQ ID NO: 74 - protein, 952 aa, Corynebacterium stationis
MDFIARHLGPDATESKDMLARVGYDSVEALVTSAIPQSISITDALNMPQALSETDAQAKLRAYADKNVVLKSFYGQGYSDTITPAVIRRGLVEDAGWYTAYTPYQPEISQGRLESLLNFQTMVQDLTGLPIANASLLDEASAVAEAVGLMSRAVKKGRRVLLDARLHPQVLTVAAERARAIDLEVEIADLSNGVVGEDLVGAVVAYTGTEGDIFDPRAVIEEIHGRGGLVSVAADLLSLLLLEGPGSFGADIVIGSSQRFGVPLFFGGPHAAFMAVTDKLKRQMPGRLVGVSVDSEGRPAYRLALQTREQHIRRERATSNICTAQALLANVAAMYAVYHGPEGLKEIANHVHSLAASFAGAVTTQGLKITSSEFFDTVTVAGVDAASIKFSLEKAGYLVRTIGEDKVSVSFGESATQGDVTVLADAFGAAAVDNADFPLPEALTRTTEVLTHEIFNSIHSETQMMRYLRKLGDKDLALDRTMIPLGSCTMKLNPTAAMEPITWPEFANVHPYSPEYATQGWRELIEELEGWLAELTGYAKVSIQPNAGSQGELAGLLAIRRYHVANGDTNRDIVLIPASAHGTNAASATLANLRVVVVKTAEDGSIDLEDLDAKIAKHGQNMAGIMITYPSTHGVFDPEVREVCDKIHAAGGQVYIDGANMNALTGWAQPGKFGGDVSHLNLHKTFTIPHGGGGPGVGPIGVAEHLIPFLPTDAAADELDPANPTPVEQGVPITASQFGSAGVLPITWAYIAMTGGEGLTSATAHAILGANYLARELSDSFPILFTGNEGLVAHECILDLRALTDASGVTAADVAKRLIDFGFHAPTLAFPVAGTLMVEPTESEDIAELDRFIEAMRTIRAEIQEIIDGKIAYEDSVIRHAPYTAPSVSSDDWEYSFSREKAAWPVPSLRLNKYFPPVRRLDEAYGDRNLVCSCPPPEAFDFDADTDSTEEA

SEQ ID NO: 75 - DNA, 2859 bp, Corynebacterium stationis
  source 1..2859: mol_type = genomic DNA
atggatttcattgcccgccaccttgggccagatgccacagaatctaaggacatgctggcgcgtgtgggttatgacagcgtagaagcgcttgtcacctcagcaatcccccagtccattagcatcacggatgcgcttaatatgccgcaggcattgagtgagaccgacgcacaagccaagcttcgcgcttacgctgataaaaatgtcgtgctgaagtctttctacggccagggctactcagacaccatcacccctgctgttattcgccgcggtttggtagaagacgctggttggtacaccgcttataccccataccagccagaaatttcccagggtcgccttgagtcgctgctgaacttccagaccatggttcaagacctcaccggcttgcctattgcgaatgcttctttgctggatgaggcatcggcagttgctgaggccgtgggtttgatgtctcgtgcggtcaagaagggccgccgcgtactgctcgacgcccgtttgcacccacaggttctcaccgtggcggcggagcgtgcccgagcaattgacctcgaagttgagattgctgacttgagcaacggcgtggttggcgaagacctcgtcggcgcagtagttgcctacaccggtacggagggcgatatttttgacccacgtgctgttatcgaagaaatccatggccgcggcggacttgtttccgtcgcggctgacttgttgtccttgctgcttctggaaggcccaggctcgttcggtgcagacattgtcattggttcctcccaacgctttggtgtgccgctcttctttggtggcccacacgctgctttcatggcagtaactgacaagctaaagcgtcagatgccaggccgtttggtcggcgtatcggtcgattctgagggccgtcctgcttaccgcttggcgctgcagactcgtgaacagcacatccgccgtgaacgcgcgacgtcaaatatttgtaccgcgcaggcacttctggccaacgtggctgccatgtacgccgtctaccacggtccagaaggcttgaaggagattgctaaccacgtgcactccttggctgcttcctttgccggtgcagttactactcagggtctgaagattacttcctcggagttcttcgacaccgttaccgttgccggcgttgatgccgcatccattaagttcagcttggaaaaggccggatacctggtgcgcaccattggcgaggataaggtttctgtctccttcggtgagtccgcaacccaaggcgatgttactgtcttggcggacgcctttggtgccgctgcagtagataatgcagatttcccactgcctgaagcactcacccgcaccaccgaggtgctcacccacgaaatctttaactccattcactccgaaacccagatgatgcgttacctgcgcaagctcggtgataaggatctggctctagatcgcaccatgattcctttgggctcatgcaccatgaagctcaacccaaccgcagccatggaaccgatcacctggccagaattcgccaatgttcacccttactcccctgaatacgcaacccagggctggcgtgagctcattgaagagttggaaggctggttggctgagctgaccggctacgccaaggtttctatccaaccaaacgctggttcccagggcgagctagctggtcttttggctatccgccgctaccacgtcgcaaatggtgacaccaaccgcgatatcgtgttgattcctgcgtccgcgcacggcaccaacgctgcctccgcgaccctggcaaatctgcgcgttgttgtggttaagaccgccgaagacggctccatcgatctggaagatctcgatgcgaagatcgccaagcatggtcagaacatggccggaatcatgatcacctacccatccactcacggcgtctttgacccagaggttcgtgaagtctgcgacaagatccatgccgctggcggccaggtctacattgatggcgcaaacatgaatgctttgactggttgggctcagccgggcaagttcggtggcgatgtctcgcacttgaacctgcacaagactttcaccattccgcacggcggtggcggcccaggtgttggaccaattggtgtcgctgagcacctcattccattcctgccaacggatgctgcagctgatgagctggatcctgctaacccaaccccagtagaacagggcgttccaattactgcttcgcagtttggttccgctggtgttctgccgattacctgggcatacatcgcaatgaccggtggcgagggtctaacctccgctactgcacacgccatcttgggtgctaactaccttgcgcgcgaactctccgattccttcccaattctgttcaccggtaatgaaggtcttgttgcgcacgagtgcattttggatctgcgcgcgctaaccgatgcctcaggcgttactgcagcagacgttgccaagcgtttgatcgactttggcttccacgctcctaccctcgcattcccagtggctggcaccttgatggtggaacctactgagtctgaggatattgctgaactggatcgtttcattgaagcaatgcgcaccatccgtgcggagattcaggaaatcatcgatggcaagatcgcatatgaagattcggtcatccgccacgcaccttacaccgcaccgtcagtctcaagcgatgattgggagtactcctttagccgtgaaaaggccgcatggccagttccttcactgcgtttgaacaagtacttcccaccggtacgccgcctggatgaagcttacggcgaccgcaacctggtgtgctcctgcccaccgccagaggcattcgacttcgatgccgacaccgattccaccgaggaggcttaa

SEQ ID NO: 76 - protein, 367 aa, Corynebacterium stationis
MSELRQSPLHAEHEKLGASFTAFGPWNMPLKYGKELDEHHAVRNAVGMFDLSHMGEIWVNGPDAAAFLSYALISNMETVKNGKAKYSMIVAEDGGIIDDLISYRFSDTKFLVVPNAGNTDVVWEAFNQRIEGFDVELNNESLDVAMIALQGPNAAKVLVEQVAEESKEEVENLPYYAATMAKVADVDTIVARTGYTGEDGFELMIYNADATKLWQLFIDQDGVTPCGLASRDSLRLEAGMPLYGNELSRDITPVEAGMGVAFKKKTADFVGAEVLRQRLEEGPKQVIKALTSSERRAARTGAEIYAGEQLVGTVTSGQPSPTLGHPIALALVDTAANLEEGAEVEVDIRGKRYPFTVTKTPFYSREK

SEQ ID NO: 77 - DNA, 1104 bp, Corynebacterium stationis
  source 1..1104: mol_type = genomic DNA
atgtcagaactacgccagtccccactgcacgcagagcacgaaaagctcggcgcatcctttaccgcttttggcccttggaatatgccactaaagtacggcaaggagctcgatgagcaccacgcagtgcgtaatgcagtcggcatgtttgacctctcgcacatgggtgagatttgggtcaacggcccagacgccgctgcatttttgtcctatgcgctgatctccaacatggagaccgtgaaaaatggcaaggcgaagtactccatgattgttgctgaagacggcggcatcatcgatgacctaatttcctaccgtttctccgataccaagttcttggtagtgccaaacgctggcaacactgatgtggtttgggaagcttttaatcagcgcattgaaggcttcgatgtagaactcaacaatgagtccttggatgttgcgatgattgccctgcagggccccaatgctgccaaggttctagttgaacaggttgctgaagagtccaaggaagaagtagaaaaccttccttactatgccgcaaccatggccaaagtcgcagacgttgacaccatcgtcgcgcgcaccggctacaccggcgaagacggcttcgagctgatgatctacaacgccgatgcgaccaagctctggcagcttttcatcgaccaagatggtgttactccatgcggtttagcttcacgcgattccttgcgcttggaagctggcatgcctttgtacggcaatgagctttcccgcgatatcacccctgtcgaggcaggcatgggtgtggcgtttaagaagaagaccgctgacttcgtcggcgccgaggtcctgcgtcaacgcttggaagaaggccctaagcaagttatcaaggctttgacctcctctgagcgccgtgcagcgcgcaccggtgctgaaatctatgccggcgagcagttggtaggcaccgtaacttcgggtcagccatcgccgacgctgggacaccctattgccctggcactggtagatactgcagcaaacctcgaagaaggcgcagaagtagaagtggatattcgcggcaagcgttaccccttcaccgttaccaagacgcctttctatagccgcgagaagtaa

SEQ ID NO: 78 - protein, 129 aa, Corynebacterium stationis
MANLPAEFTYSEDHEWINAAQDAIVGKTVRIGITSVAADRLGEVVFAELPAVGDSVTAGETCGEVESTKSVSDLYSPVTGTVTAVNETVHDDYEIINNDPFGEGWLFEVEVEELGEVMTADEYAAENGI

SEQ ID NO: 79 - DNA, 390 bp, Corynebacterium stationis
  source 1..390: mol_type = genomic DNA
atggctaacctacctgcagaatttacttactccgaagaccacgagtggattaacgccgctcaggacgcaatcgttggcaaaactgttcgcatcggcatcacttctgttgccgcagaccgtcttggtgaggttgtcttcgctgagcttccagcagttggcgatagcgtcactgcaggtgaaacctgtggtgaggttgaatccaccaagtccgtttctgacctgtacagccctgtcaccggtaccgtgaccgctgtgaacgagacagtgcacgatgattatgaaatcatcaacaatgatcctttcggtgaaggttggctgtttgaggtcgaggttgaagaactcggcgaggttatgaccgctgatgaatacgcggcagaaaacggcatctaa

SEQ ID NO: 80 - protein, 433 aa, Corynebacterium stationis
MTTQNSSDAQYQEMRDLDPEVYAAINGEIARQRDTLEMIASENFVPRAVLQAQGSVLTNKYAEGYPGRRYYGGCEHVDIVEDLARDRAKALFGAEFANVQPHSGAQANAAVLASLINPGDKILGLSLAHGGHLTHGMKLNFSGKLYEVAAYEVDAETNRIDMDKLREQAIAEKPQVIIAGWSAYPRTLDFEAYRSIADEVGAYLWTDMAHFAGLVAADLYPNPVPHSDIVSTTVHKTLGGPRSGMILAKQDYAKKLNSAVFPGQQGGPLMHVVAAKAIAMKVAASEEFRDRQVRTLEGAKILAERLTTPEAKAAGVDVLTGGTDVHLVLADLRNSEMDGQQAEDLLHEVGITVNRNAVPNDPRPPMVTSGLRIGTSALATRGLDAEAFTEVADIIGTALTDGKNADTQKLRARVDKLAEQFPLYEGLEDWKIV

SEQ ID NO: 81 - DNA, 1302 bp, Corynebacterium stationis
  source 1..1302: mol_type = genomic DNA
atgactacccagaattcttccgatgctcagtaccaggaaatgcgtgacttagacccagaggtctatgcagcaattaacggtgaaattgctcgtcagcgcgataccctggagatgattgcgtcggagaactttgttcctcgtgcagtcttgcaggcacagggttccgtccttaccaacaagtacgcagagggctacccaggtcgccgctactacggtggatgtgagcacgtcgatatcgtcgaagatctggcgcgtgaccgcgctaaggctctgttcggcgctgagtttgccaatgtacagccacactccggtgcacaggcaaacgctgccgtccttgcttctcttatcaacccaggcgataagatcttgggcctttctttggctcacggtggtcacctgacccacggcatgaagctgaacttctccggcaagctctacgaagtagctgcctacgaagtcgatgcagaaaccaaccgtatcgacatggacaagctgcgtgagcaggctattgcagaaaagccacaggtcatcatcgctggctggtctgcatacccacgcactctggattttgaagcataccgttccatcgcggatgaagtgggggcttacctgtggaccgatatggcacactttgctggtctcgttgccgctgatctgtacccaaatccagttccacactctgacattgtttccaccaccgtgcacaagaccctgggcggtcctcgctccggcatgatcctggctaagcaggactacgctaagaagctcaactctgcagtcttcccaggccagcagggtggccctttgatgcatgtggttgcagcgaaggcaattgccatgaaggttgctgcttccgaagaattccgtgaccgtcaggtccgtactctggaaggcgcgaagattcttgctgagcgcttgaccactcctgaggcaaaggcagcaggcgttgacgttctcactggcggcaccgacgtgcacttggttcttgcggacctgcgcaattctgagatggatggccagcaggcagaagacctcctgcacgaggtcggcatcaccgttaaccgcaacgcggttccaaacgatccacgtccaccaatggtgacctctggtctgcgtatcggtacttccgctctggctacccgcggcctggatgcagaagcattcaccgaggtggcagacatcatcggcaccgcgcttaccgatggcaagaacgccgatacccagaagctgcgcgcacgcgtggacaagcttgctgagcagttcccactctacgagggcttggaagactggaagatcgtctaa

SEQ ID NO: 82 - protein, 422 aa, Corynebacterium stationis
LESYIGSPLTSNAVRVLMLGGGELAKGLVGAFQNLGLEVHVVDRYEGSPAQQVAHFSYTADIDDEKAVLDLVEHIKPAYVVPEIEGVADEALHALHDDSAVTVVPTARACELTSDRKKLREVAESLGLPTTAYKVVETFDALKEAVNELGLPCIIKPDVATSGRGHVLVKDEDQLKDAWDNVRRGKKNSWVVAERFVDFDYEVIIMAVRSIDPETGKLATWFSEPIGYEHARGNLVDCWQPKTMSQRAFENARSVAARISNELGGRGIFAVELFVAGDDIYFSSVTPRPSDKAMLTEATQRFSQYELHARAILGLPIDITLVSPGASSLLHATEEIDEVTYSGVEEALQVAETDVRLFGKPSAYPGRRMGLIMATADDVSEARDRAAIAASKITISAAPRLVPEPELTSEKELSPDEVEISE

SEQ ID NO: 83 - DNA, 1269 bp, Corynebacterium stationis
  source 1..1269: mol_type = genomic DNA
ttggagtcttatatcggtagccccctgacctcgaatgctgttcgggttctcatgctcggcggcggtgagctggccaaaggtttggtgggcgcgtttcagaatttgggcttggaagtccacgttgtcgaccgctatgaggggtctccagcacagcaggttgcacactttagctacaccgcagatatcgatgatgaaaaggccgtgctcgatttagttgagcacatcaagccggcttatgtcgtgccagaaatcgagggcgtagcagatgaggctttgcatgcgcttcacgatgactccgctgtcaccgttgtgcccaccgcccgggcgtgtgagcttaccagcgaccggaagaagctacgcgaagtcgcagaaagcctcggcttgccgacgaccgcgtacaaggtcgtagaaaccttcgacgctttgaaagaagcggtgaacgagctcggtttgccgtgcattattaagccggatgttgcaacctctggacgcgggcatgtgctggtcaaagacgaagaccaactcaaagacgcgtgggataatgtgcgtcgcggcaagaagaactcctgggttgtcgccgaacgctttgtggattttgactatgaagtcatcatcatggcggtgcgctcgattgacccggaaacgggcaagctggcaacgtggttctcagagccgattggttatgagcatgcgcgcggcaacctcgtggactgctggcagccaaagacgatgagccagcgtgcttttgaaaatgcacgttcggttgcagcgcgtatttctaacgaactcggcggccgcggcatcttcgcggtggagctgtttgtcgcgggcgacgatatctacttctcctcggtgaccccgcgtccttctgataaagcgatgctgaccgaagccacccaacgcttttcgcagtatgaattgcacgcgcgcgccattttgggcctgccgatcgacatcacgcttgtctcaccgggcgctagctctttgttgcacgcgaccgaagagatcgacgaagttacctactcgggcgttgaagaagccctgcaggttgcagaaaccgatgtgcgcctattcggcaagccttcggcataccctggccgacgcatggggttgatcatggccaccgccgacgatgtctccgaagcacgcgaccgcgctgcgatcgcggcatcgaagatcacgattagcgccgccccaaggttagttcctgaaccagaactaacctctgaaaaagagttatcccccgatgaggtcgaaatctccgagtaa